European Patent Specification EP 3 611 182 B1, published February 14, 2024. Title: Peptides having cytoprotective effects against environmental pollutants and use thereof. Applicant: CAREGEN CO., LTD. The sequence listing filed with the application follows.

SEQUENCE LISTING (13 sequences)

SEQ ID NO: 1 - protein, 7 aa, Artificial Sequence
  Artificial Sequence
KWGGGRY

SEQ ID NO: 2 - protein, 7 aa, Artificial Sequence
  Artificial Sequence
ILGRWCG

SEQ ID NO: 3 - protein, 6 aa, Artificial Sequence
  Artificial Sequence
DVENTS

SEQ ID NO: 4 - DNA, 21 bp, Artificial Sequence
  CYP1A1_F
ggatctttctctgtaccctgg

SEQ ID NO: 5 - DNA, 20 bp, Artificial Sequence
  CYP1A1_R
agcatgtccttcagcccaga

SEQ ID NO: 6 - DNA, 21 bp, Artificial Sequence
  TNF-a_F
cgtcagccgattrtgctatct

SEQ ID NO: 7 - DNA, 20 bp, Artificial Sequence
  TNF-a_R
cggactccgcaaagtctaag

SEQ ID NO: 8 - DNA, 20 bp, Artificial Sequence
  IL-6_F
aaagaggcactgccagaaaa

SEQ ID NO: 9 - DNA, 20 bp, Artificial Sequence
  IL-6_R
atctgaggtgcccatgctac

SEQ ID NO: 10 - DNA, 20 bp, Artificial Sequence
  IL-1b_F
ttcgacacatgggataacga

SEQ ID NO: 11 - DNA, 20 bp, Artificial Sequence
  IL-1b_R
tctttcaacacgcaggacag

SEQ ID NO: 12 - DNA, 21 bp, Artificial Sequence
  COX-2_F
atcattcaccaggcaaattgc

SEQ ID NO: 13 - DNA, 21 bp, Artificial Sequence
  COX-2_R
ggcttcagcataaagcgtttg